European Patent Application EP 4 623 998 A2, published October 1, 2025. Title: TREATING METASTATIC CANCER AND MODEL SYSTEMS FOR METASTATIC DISEASE. Applicant: MEMORIAL SLOAN-KETTERING CANCER CENTER. Application EP. The sequence listing filed with the application follows.

SEQUENCE LISTING (6 sequences)

SEQ ID NO: 1 - DNA, 58 bp, synthetic construct
  misc_feature 1..58: note = RNAi hairpin
  source 1..58: mol_type = other DNA
ccggacgggcaacaacagcaactttctcgagaaagttgctgttgttgcccgttttttg

SEQ ID NO: 2 - DNA, 21 bp, synthetic construct
  misc_feature 1..21: note = RNAi target
  source 1..21: mol_type = other DNA
acgggcaacaacagcaacttt

SEQ ID NO: 3 - DNA, 58 bp, synthetic construct
  misc_feature 1..58: note = RNAi hairpin
  source 1..58: mol_type = other DNA
ccggccacttgtttaaggagaggatctcgagatcctctccttaaacaagtggtttttg

SEQ ID NO: 4 - DNA, 21 bp, synthetic construct
  misc_feature 1..21: note = RNAi target
  source 1..21: mol_type = other DNA
ccacttgtttaaggagaggat

SEQ ID NO: 5 - DNA, 58 bp, synthetic construct
  misc_feature 1..58: note = RNAi hairpin
  source 1..58: mol_type = other DNA
ccgggccaatgcctacatctacgttctcgagaacgtagatgtaggcattggctttttg

SEQ ID NO: 6 - DNA, 21 bp, synthetic construct
  misc_feature 1..21: note = RNAi target
  source 1..21: mol_type = other DNA
gccaatgcctacatctacgtt